European Patent Specification EP 3 484 276 B1, published January 17, 2024. Title: ToLCNDV resistant melon plants. Applicant: NUNHEMS B. V. The sequence listing filed with the application follows.

SEQUENCE LISTING (24 sequences)

SEQ ID NO: 1 - DNA, 200 bp, Cucumis melo
agctggtgcaaagctggcattcaaatcgaatgaagaaatagcagtacaagtgaagtcaattccactagatgaagtaatcccggattcagaacgagtgcttctaataaaaatcgatgttcaaggctgggaatatcatgtgctaaaaggggcaaagagaattttgtcaaggaagggcactgaagctccatatctcatctatg

SEQ ID NO: 2 - DNA, 1145 bp, Cucumis melo
ttgtaatcatggccattgcctgatytgcagaatgtggcgtcttgattgggcacggtctggatgaagttactccaaagcttgtggaagttaatgggttcttctcttcaccrtctgrtctccttcccatcgacaatgtggtttcttcttcaaacacaaaagaaacccctgttgaagctgtagaagaaagctgtgagttcttttctccactcagttctaggtttagttttttatttgttttttttttcttttttcctttttacttgctttgagctgtaggacacaacacaaaatgataagaacaaaaatcaatctatgttattgttgtcattgtctcgcctgcctcttcaaggtaactaggctataacactgatccaaaatgtataatctttattgctaagtaacttatattgcaaagattgggatggaataggagcataggttgcatctaatagttttgtccaactttggttatagtttcagccagtttgttcagatgaaattcttagtgattatcactaatggaattgtttttataaatgttgtaggtgttgaaagaagtgaagaatatgaaaaggaaagcaggggaaccgagaaggctgaaatcttaccgacaaaagcaacatctgaagcaggttctgaagtccaacctgtttccagtgattctgctcagatggtacccaatatgttggagctcggtgatgcttataagctagctgtaggtgctagaggaggaagacaattgtctggcaagcttttggaacaatggatygggaaggaatcttcaaaagttagtgaagatctgaagcttctcttgacacaactctcatttaatcgtttgaatgaccaatcacgggagatgagtccaaggctgtccgtaaatggagacgaggtgaggaactttgattacttgagygctgttgggatgcaaatgctacaaaaaaggwtttcgcttgaaagaaatgagtccggtgtagaatctttagatggaagcataattagtgaaatcgatggggaaaacatggctgataggttgaaacgacagattgagtatgataagaaggttmtgarttctttatacaaggaattggaggaagaaagaaatgcatccgcaattgctgcaaatcaggcaatggccatgattacaa

SEQ ID NO: 3 - DNA, 168 bp, Cucumis melo
agacggcgtacatgcagcattctgttaccccgcgatgcccagcgatgaaacaactcctttgcatccttatggtccagaggttccagatcatacgactcaccaaatgcaggaaacttaaatctagaggtgaccaaaattttgcagttgggtaatcgggagaacttttca

SEQ ID NO: 4 - DNA, 468 bp, Cucumis melo
ggagkcttcatccgtctttaccttcctcacttttttacctaaccaagttacgtcttgtaggttgcaagataacaaatttggatttcttagaaacaattgtttatgttgccccttcrttgaaagagttggacttgtccgaaaacaacttttgtagamtaccctcrtgtattattaattttaaatccctgaaatatctttatacaatggattgtgagttgctygaagaaatttcaaaggttccagaaggtgtaatttgtacgagtgccgcaggatgcaaatcattggctagatttcccgacaacttagctgatttcatatcttgtggtaattctgcggtgcgtaccatatctctttctcatgacttcaccattatctctagctcatgtatatttaatttcattcatataatatatattacttataactatttactgatctcatggtgcaggaatgttgtaaaggtggatg

SEQ ID NO: 5 - DNA, 1047 bp, Cucumis melo
tgcaggtagtcaaaccaattgataatatttgctcaccatcaaaattggtaaccatagacatagaytgaccaagcccaggcaaaacggcatcatctttttgttttctatcattactattctgattacccaaaagaaatcttctttttgtacttggagagaaataatccccgtctgcacattgcatggaaggtgtgctgtcatgagcatcagcattacacacaccagaattagatttcttgctagccaagatttcacaaccaccaagagaagcaggacctacgcctggggtctctgcctyagaaagccaagsatcaaagcacacttgtgaaggacctgaaactgtctcagatccagggatttctcctacattgggtaagctagcctgttcaaagccatcacacacatctacaagcggcagtctaccatacatggaactattagaataagcaggcttattttcataaaacacattaacgcttgcatttggattagttaaacatggcatcaaatgggaagaatcccgaaatctcaagctgttctcattggaccgcagcactccagaattcaagtctcttgaccatacttttttttgcctgctatcaacagtaaaattttgagctttaccatatccacagtcaagtggctcatttcgagagttacgcttcctcctcattaaatcacktacagaacggccttccctggagttatgtgtgcctgtacctgcatttcgtaatgtaacatccacctgccctccatcttcacttgaaaagcaactaatgaactcagaatctttggtcgaacttgtccatatgtcaggcctgcaagaattgacacacgtcgaatctgtattcactttctcagcctcatgaaaaggtaaagatccccaaaatgatttctctttcttgtgactgcaagaacctgaatcaatgccatgcaataatattgcaagtttggaagatctttcattctcaacattaagatctctatcaggtgagttttcagtcgaccctccagaagaagagaacatatcatctgcakgtacgcagt

SEQ ID NO: 6 - DNA, 1118 bp, Cucumis melo
gcgtacmtgcaggcaaagaatggcacagtacagtaatggtagctcatctgttcatcaaggagaatcaagctgcctcagccattcagtatcggttccacccctgatcatctcctacaatgatcgcattcgtcctctccttgatgctgttgacaagcttcgtcacctcatgatcatgagagaaggcatccaactgcctaccatagttgttgttggtgatcagtcawccggtaagtcaagtgtcctcgagtcgttggctgggatcagcctacctcgaggtcagggcatctgcaccagggtccctctgataatgaggctccaaaaccatcctgatcccgaacccgagcttgttttggagtacaatgggaaaaagatccacaccgacgaatccttcattgctgaagacatctgtacagctacagaggagattgctggcagtggcaaaggaatatcgaaagcgccattgactttgattgtgaagaaaaatggtgttcctgatcttacaatggttgatctccctggaattacragagtgcctgttaaagatcagcctgaagacatttatgaccaaataaaagatataatcatggaacatatcaagccagaagagagcatcatcttgaatgtcttgtctgcgacggttgattttccaacttgtgaatcgatacggatgtctcaaagtgtcgacaagacgggaatgagaacgttggcagttgtgactaagtctgacaaggcaccagaaggcctacacgagaaggtcaccrcggatgatgtcagtatcggccttggttatgtttgcgttaggaaccgaattggcaatgagacatatgaggaagctcgggttgcagaagccaaattgttttcaactcatcctcttctctccaaaattgacaaatctgttgtgggcattccagtcttggctcagaagttggtgcaaattcaagcaggtacccaaactaattcctgactcaaaagctaggttccgttagataaccattttgttttagaaaatcaagtttattttctctaaatmgtgtaccatgattttcatctttcttaaataaaaaagttgmattcttwactaaattttaaaagcaaaaacaagttttaatacttttttt

SEQ ID NO: 7 - DNA, 43 bp, Artificial Sequence
  KASP-assay FAM SNP_01
gaaggtgaccaagttcatgctccggattcagaacgagtgcttc

SEQ ID NO: 8 - DNA, 44 bp, Artificial Sequence
  KASP-assay VIC SNP_01
gaaggtcggagtcaacggattcccggattcagaacgagtgcttt

SEQ ID NO: 9 - DNA, 29 bp, Artificial Sequence
  KASP-assay common primer SNP_01
atgatattcccagccttgaacatcgattt

SEQ ID NO: 10 - DNA, 45 bp, Artificial Sequence
  KASP-assay FAM SNP_02
gaaggtgaccaagttcatgctcggactcatttctttcaagcgaac

SEQ ID NO: 11 - DNA, 46 bp, Artificial Sequence
  KASP-assay VIC SNP_02
gaaggtcggagtcaacggattccggactcatttctttcaagcgaaa

SEQ ID NO: 12 - DNA, 27 bp, Artificial Sequence
  KASP-assay common primer SNP_02
ygctgttgggatgcaaatgctacaaaa

SEQ ID NO: 13 - DNA, 43 bp, Artificial Sequence
  KASP-assay FAM SNP_03
gaaggtgaccaagttcatgctgatctggaacctctggaccatg

SEQ ID NO: 14 - DNA, 45 bp, Artificial Sequence
  KASP-assay VIC SNP_03
gaaggtcggagtcaacggattatgatctggaacctctggaccata

SEQ ID NO: 15 - DNA, 26 bp, Artificial Sequence
  KASP-assay common primer SNP_03
ccagcgatgaaacaactcctttgcat

SEQ ID NO: 16 - DNA, 50 bp, Artificial Sequence
  KASP-assay FAM SNP_04
gaaggtgaccaagttcatgctaaattacaccttctggaacctttgaaatt

SEQ ID NO: 17 - DNA, 45 bp, Artificial Sequence
  KASP-assay VIC SNP_04
gaaggtcggagtcaacggattacaccttctggaacctttgaaatc

SEQ ID NO: 18 - DNA, 30 bp, Artificial Sequence
  KASP-assay common primer SNP_04
ctttatacaatggattgtgagttgctygaa

SEQ ID NO: 19 - DNA, 46 bp, Artificial Sequence
  KASP-assay FAM SNP_05
gaaggtgaccaagttcatgctggctgagaaagtgaatacagattcg

SEQ ID NO: 20 - DNA, 47 bp, Artificial Sequence
  KASP-assay VIC SNP_05
gaaggtcggagtcaacggattaggctgagaaagtgaatacagattca

SEQ ID NO: 21 - DNA, 25 bp, Artificial Sequence
  KASP-assay common primer SNP_05
gtccatatgtcaggcctgcaagaat

SEQ ID NO: 22 - DNA, 48 bp, Artificial Sequence
  KASP-assay FAM SNP_06
gaaggtgaccaagttcatgctatcaaagtcaatggcgctttcgatatt

SEQ ID NO: 23 - DNA, 46 bp, Artificial Sequence
  KASP-assay VIC SNP_06
gaaggtcggagtcaacggattcaaagtcaatggcgctttcgatatc

SEQ ID NO: 24 - DNA, 23 bp, Artificial Sequence
  KASP-assay common primer SNP_08
gaggagattgctggcagtggcaa